European Patent Specification EP 3 524 604 B1, published March 29, 2023. Title: COMPOUNDS THAT EXPAND HEMATOPOIETIC STEM CELLS. Applicant: NOVARTIS AG THE SCRIPPS RESEARCH INSTITUTE. Application EP19164770.0. The sequence listing filed with the application follows.

SEQUENCE LISTING (4 sequences)

SEQ ID NO: 1 - DNA, 61 bp, Homo sapiens
gcggcatagagaccgacttaatttcaagagaattaagtcggtctctatgccgcttttttgg

SEQ ID NO: 2 - DNA, 65 bp, Homo sapiens
cgcgccaaaaaagcggcatagagaccgacttaattctcttgaaattaagtcggtctctatgccgc

SEQ ID NO: 3 - DNA, 61 bp, Homo sapiens
ggcttctttgatgttgcattaattcaagagattaatgcaacatcaaagaagccttttttgg

SEQ ID NO: 4 - DNA, 65 bp, Homo sapiens
cgcgccaaaaaaggcttctttgatgttgcattaatctcttgaattaatgcaacatcaaagaagcc